European Patent Application EP 4 361 275 A1, published May 1, 2024. Title: 22056WO. Applicant: Amano Enzyme Inc. The sequence listing filed with the application follows.

SEQUENCE LISTING (3 sequences)

SEQ ID NO: 1 - protein, 614 aa, Chrysocorona lucknowensis
MKTFIGAVALMLGAVVPRVIAAPPGNAIQRDLLVPLEERQDTARPPRQISCHTPSNRACWTTGFNINTDYEVSTPNTGVVRPYTLTLTEVDNWTGPDGVVKNKVMLVNGPTIFADWGDTIQVTVINNLLTNGTSIHWHGLRQKDTNLHDGANGVTECPIKPGGGRRVYRFRAQQYGTSWYHSHFSAQYGNGVVGTIQINGPASLPYDIDLGVFPLQDYYYRSADELVHFTMNNGPPFSDNVLFNGTAKHPTTGAGQYANVTLTPGKRHRLRLINTSTENHFQVSLVNHTMTIIAADLVPVNAMTVDSLFLGVGQRYDVTIDANRTPGNYWFNVTFGGGNLCGGSNHPNPAAIFHYAGAPGGLPTDRGTPPVDHQCLDLPNLTPVVTRNVPVSGFVKRPGNTLPVHLDTTGTPLFVWKVNGSAINVDWNKPVLEYVLTQNTSYPASNNIVQVDAVDQWTYWLVENDPDAPFTLPHPMHLHGHDFVVLGRSPDVPAATQQRFVFDPAVDLPRLRGTNPVRRDVTMLPPKGWLLLAFKTDNPGAWLFHCHIAWHVSGGLSVQFLERPNELRQGISQADRDDFNRVCNDWRAYWPTNPFPKIDSGLRHRFVEEMQYNI

SEQ ID NO: 2 - DNA, 1845 bp, Chrysocorona lucknowensis
atgaagaccttcatcggcgccgtggcgctcatgctcggtgctgttgtccccagggtcatcgccgctcctccgggcaacgccatccagagagacctcctcgtgccccttgaggagagacaggacacggccagacctcctcgtcagatcagctgccacaccccgagcaaccgagcgtgctggaccactggcttcaacatcaacactgactatgaagtcagcactcccaacactggcgtcgttcggccttacaccctcactctgacggaggtggacaactggaccggtccagacggcgttgtcaagaacaaggtcatgctggtcaacggcccgactatcttcgctgactggggtgacaccatccaagtcaccgtcatcaacaatctcctcaccaacggcacctccatccactggcacggcttgcgccagaaagataccaacctgcacgatggagccaatggtgttactgaatgccctataaaaccagggggaggcagaagggtgtaccggttccgcgcccagcagtacgggacgagctggtaccactcgcacttctcggcccagtacggcaacggcgtggtcgggaccatccagatcaacgggccggcctcactcccttacgatatagatctaggcgtctttccgctgcaagactactactaccgcagcgctgacgagcttgtccacttcaccatgaacaacggacccccgttcagcgacaacgtcctcttcaatggcacggccaagcaccccaccacgggcgccggccagtacgcaaacgtgaccctgacgccgggcaagcgccatcgcctgcgcctgatcaacactagtacagaaaaccattttcaggtgagcctagttaaccacaccatgaccatcattgcggccgacctggtccccgtcaacgccatgacggtcgacagcctgttcctcggtgtgggccagcgctacgacgtgaccatcgacgccaaccgcacaccgggcaactactggttcaacgtgacatttggcggcggcaacctctgcggcggctccaaccaccccaacccggcggccatcttccactacgccggcgcccccggcggcctgccgaccgaccgcggcacgcccccggtcgaccaccagtgcctcgacctgcccaacctgacgcccgtcgtcacgcgcaatgtgcccgtcagcgggttcgtcaagaggcccggcaacaccctgcccgtccacctggacactaccggcaccccgctgtttgtgtggaaggtgaacgggagcgcgatcaatgtcgactggaacaagccggtgctggaatatgtcctgacgcagaacacgagctatccggcgagcaataacatcgtgcaggttgacgcggtcgaccagtggacctactggctcgtcgagaacgacccggatgcaccattcactctgccgcacccgatgcacttgcacggccacgacttcgtcgtcctcggccgctccccggacgtcccggccgcgacgcagcagcgcttcgtgttcgatccggccgtcgacctgccgcggctgcgcgggaccaacccggtccggcgcgacgtcaccatgctgccgcccaagggctggctgctgctggccttcaagacggacaacccgggcgcctggctgttccactgccacatcgcctggcatgtgtcgggcgggctgagcgtgcagttcctcgagcggcccaacgagctgcgccagggcatctcgcaggccgaccgggatgatttcaatcgcgtctgcaacgactggcgcgcgtactggccgacgaatccgttccccaagatcgattcagggctgaggcaccggttcgttgaggagatgcaatacaacatatag

SEQ ID NO: 3 - DNA, 2392 bp, Chrysocorona lucknowensis
atgaagaccttcatcggcgccgtggcgctcatgctcggtgctgttgtccccagggtcatcgccgctcctccgggcaacgccatccagagagacctcctcgtgccccttgaggagagacaggacacggccagacctcctcgtcagatcagctgccacaccccgagcaaccgagcgtgctggaccactggcttcaacatcaacactgactatgaagtcagcactcccaacactggcgtcgttcggcctgtaagaggctcctctctgcaggggaacagctggatgctaagtacaggcagtacaccctcactctgacggaggtggacaactggaccggtccagacggcgttgtcaagaacaaggtcatgctggtcaacggtatgtcatattgctcagtggcattcttatcttgactaatacatttcgctgcaggcaagattcttggtgcgcctaacctccccctttcaccccgcctcctagggttagggttaacacccttcccctccggcccccggacgcggacccggatccttagccacgacctcaccgggttgaactacatatactgacttgcttaggcccgactatcttcgctgactggggtgacaccatccaagtcaccgtcatcaacaatctcctcaccaacgggtacgtccctcgccgcatcagaagttcacccctaacttccatgacacagcacctccatccactggcacggcttgcgccagaaagataccaacctgcacgatggagccaatggtgttactgaatgccctataaaaccagggggaggcagaagggtgtaccggttccgcgcccagcagtacgggacgagctggtaccactcgcacttctcggcccagtacggcaacggcgtggtcgggaccatccagatcaacgggccggcctcactcccttacgatatagatctaggcgtctttccgctgcaagactactactaccgcagcgctgacgagcttgtccacttcaccatgaacaacggacccccgttcagcgacaacgtcctcttcaatggcacggccaagcaccccaccacgggcgccggccagtacgcaaacgtgaccctgacgccgggcaagcgccatcgcctgcgcctgatcaacactagtacagaaaaccattttcaggtgagcctagttaaccacaccatgaccatcattgcggccgacctggtccccgtcaacgccatgacggtcgacagcctgttcctcggtgtgggccagcgctacgacgtgaccatcgacgccaaccgcacaccgggcaactactggttcaacgtgacatttggcggcggcaacctctgcggcggctccaaccaccccaacccggcggccatcttccactacgccggcgcccccggcggcctgccgaccgaccgcggcacgcccccggtcgaccaccagtgcctcgacctgcccaacctgacgcccgtcgtcacgcgcaatgtgcccgtcagcgggttcgtcaagaggcccggcaacaccctgcccgtccacctggacactaccggcaccccgctgtttgtgtggaaggtgaacgggagcgcgatcaatgtcgactggaacaagccggtgctggaatatgtcctgacgcagaacacgagctatccggcgagcaataacatcgtgcaggttgacgcggtcgaccaggtgggttcccttcgtgcttgggtgccatcgggggtaagagcagaagactgacgaacctcgcagtggacctactggctcgtcgagaacgacccggatgcaccattcactctgccgcacccgatgcacttgcacgtaagcactccttttccttgaacttcccccgtccattcaccttggctcctgctcccaacatgcataccgacacctgatggtggttcagggccacgacttcgtcgtcctcggccgctccccggacgtcccggccgcgacgcagcagcgcttcgtgttcgatccggccgtcgacctgccgcggctgcgcgggaccaacccggtccggcgcgacgtcaccatgctgccgcccaagggctggctgctgctggccttcaagacggacaacccgggcgcctggctgttccactgccacatcgcctggcatgtgtcgggcgggctgagcgtgcagttcctcgagcggcccaacgagctgcgccagggcatctcgcaggccgaccgggatgatttcaatcgcgtctgcaacgactggcgcgcgtactggccgacgaatccgttccccaagatcgattcagggctgaggcaccggttcgttgaggagagtgagtggatggtgagggcttgactgttgtgatgaagggaaaggtaatggtgaggtcttgtagacagagtataacccttgtgtgattgttaaggtagtgcaatacaacatatag